European Patent Application EP 4 706 681 A2, published March 11, 2026. Title: CHAPERONIN-CONTAINING TCP-1 INHIBITORS FOR THE TREATMENT OF CANCER. Applicant: UNIVERSITY OF CENTRAL FLORIDA RESEARCH FOUNDATION, INC. The sequence listing filed with the application follows.

SEQUENCE LISTING (29 sequences)

SEQ ID NO: 1 - protein, 20 aa, synthetic construct
  REGION 1..20: note = Synthetic construct
VTIFVAGVLTASLTIWKKMG

SEQ ID NO: 2 - protein, 10 aa, synthetic construct
  REGION 1..10: note = Synthetic construct
ASLTIWKKMG

SEQ ID NO: 3 - protein, 10 aa, synthetic construct
  REGION 1..10: note = Synthetic construct
VTIFVAGVLT

SEQ ID NO: 4 - protein, 7 aa, synthetic construct
  REGION 1..7: note = Synthetic construct
VTIFVAG

SEQ ID NO: 5 - protein, 5 aa, synthetic construct
  REGION 1..5: note = Synthetic construct
IFVAG

SEQ ID NO: 6 - protein, 6 aa, synthetic construct
  REGION 1..6: note = Synthetic construct
IWKKMG

SEQ ID NO: 7 - protein, 8 aa, synthetic construct
  REGION 1..8: note = Synthetic construct
DYKDDDDK

SEQ ID NO: 8 - DNA, 20 bp, synthetic construct
  misc_feature 1..20: note = Synthetic construct
  source 1..20: mol_type = other DNA
tctggtaccgagctcccgaa

SEQ ID NO: 9 - DNA, 19 bp, synthetic construct
  misc_feature 1..19: note = Synthetic construct
  source 1..19: mol_type = other DNA
gatttgcccaactggtcgg

SEQ ID NO: 10 - DNA, 23 bp, synthetic construct
  misc_feature 1..23: note = Synthetic construct
  source 1..23: mol_type = other DNA
atggagaacttccaaaaggtgga

SEQ ID NO: 11 - DNA, 20 bp, synthetic construct
  misc_feature 1..20: note = Synthetic construct
  source 1..20: mol_type = other DNA
caggcggattttcttaagcg

SEQ ID NO: 12 - DNA, 18 bp, synthetic construct
  misc_feature 1..18: note = Synthetic construct
  source 1..18: mol_type = other DNA
gcgtccatgcggaagatc

SEQ ID NO: 13 - DNA, 17 bp, synthetic construct
  misc_feature 1..17: note = Synthetic construct
  source 1..17: mol_type = other DNA
atggccagcgggaagac

SEQ ID NO: 14 - DNA, 21 bp, synthetic construct
  misc_feature 1..21: note = Synthetic construct
  source 1..21: mol_type = other DNA
gccagccttgggacaataatg

SEQ ID NO: 15 - DNA, 21 bp, synthetic construct
  misc_feature 1..21: note = Synthetic construct
  source 1..21: mol_type = other DNA
agtttgggtaaacccggtcat

SEQ ID NO: 16 - DNA, 21 bp, synthetic construct
  misc_feature 1..21: note = Synthetic construct
  source 1..21: mol_type = other DNA
ggaggctattctgcccatttg

SEQ ID NO: 17 - DNA, 21 bp, synthetic construct
  misc_feature 1..21: note = Synthetic construct
  source 1..21: mol_type = other DNA
gaggctgctggttttccacta

SEQ ID NO: 18 - DNA, 19 bp, synthetic construct
  misc_feature 1..19: note = Synthetic construct
  source 1..19: mol_type = other DNA
acctgcaaccgacgattct

SEQ ID NO: 19 - DNA, 19 bp, synthetic construct
  misc_feature 1..19: note = Synthetic construct
  source 1..19: mol_type = other DNA
caggcttcttgggcgtctg

SEQ ID NO: 20 - DNA, 18 bp, synthetic construct
  misc_feature 1..18: note = Synthetic construct
  source 1..18: mol_type = other DNA
tgagccgcgactgtgatg

SEQ ID NO: 21 - DNA, 23 bp, synthetic construct
  misc_feature 1..23: note = SEQ ID NO: 22
  source 1..23: mol_type = other DNA
gtctcggtgacaaagtcgaagtt

SEQ ID NO: 22 - DNA, 22 bp, synthetic construct
  misc_feature 1..22: note = Synthetic construct
  source 1..22: mol_type = other DNA
gaaggtgaaggtcggagtcaac

SEQ ID NO: 23 - DNA, 22 bp, synthetic construct
  misc_feature 1..22: note = Synthetic construct
  source 1..22: mol_type = other DNA
tggaagatggtgatgggatttc

SEQ ID NO: 24 - DNA, 21 bp, synthetic construct
  misc_feature 1..21: note = Synthetic construct
  source 1..21: mol_type = other DNA
tcagtcggtggtcatctttgg

SEQ ID NO: 25 - DNA, 23 bp, synthetic construct
  misc_feature 1..23: note = Synthetic construct
  source 1..23: mol_type = other DNA
cctccaggtatcttttccactct

SEQ ID NO: 26 - DNA, 20 bp, synthetic construct
  misc_feature 1..20: note = Synthetic construct
  source 1..20: mol_type = other DNA
cagaggtgattctgcgtgtg

SEQ ID NO: 27 - DNA, 20 bp, synthetic construct
  misc_feature 1..20: note = Synthetic construct
  source 1..20: mol_type = other DNA
tgtcgtcgtcgtccttgtag

SEQ ID NO: 28 - DNA, 20 bp, synthetic construct
  misc_feature 1..20: note = Synthetic construct
  source 1..20: mol_type = other DNA
gttggagagaagccacgaag

SEQ ID NO: 29 - DNA, 20 bp, synthetic construct
  misc_feature 1..20: note = Synthetic construct
  source 1..20: mol_type = other DNA
gttgccagagcctttcagtc